European Patent Specification EP 3 052 517 B1, published July 19, 2023. Title: MOSAIC CONSERVED REGION HIV IMMUNOGENIC POLYPEPTIDES. Applicant: Los Alamos National Security, LLC Isis Innovation Limited Korber, Bette T.M. Hanke, Tomas McMichael, Andrew. The sequence listing filed with the application follows.

SEQUENCE LISTING (39 sequences)

SEQ ID NO: 1 - protein, 86 aa, Artificial Sequence
  Mos.Env.2.1.516-601 peptide
GFLGAAGSTMGAASITLTVQARLLLSGIVQQQNNLLRAIEAQQHLLQLTVWGIKQLQARVLAVERYLKDQQLLGIWGCSGKLICTT

SEQ ID NO: 2 - protein, 231 aa, Artificial Sequence
  Mos.Gag.2.1.133-363 peptide
PIVQNLQGQMVHQAISPRTLNAWVKVIEEKAFSPEVIPMFTALSEGATPQDLNTMLNTVGGHQAAMQMLKDTINEEAAEWDRVHPVHAGPIAPGQMREPRGSDIAGTTSNLQEQIGWMTSNPPIPVGDIYKRWIILGLNKIVRMYSPVSILDIRQGPKEPFRDYVDRFFKTLRAEQATQEVKNWMTDTLLVQNANPDCKTILRALGPGATLEEMMTACQGVGGPGHKARVL

SEQ ID NO: 3 - protein, 69 aa, Artificial Sequence
  Mos.Gag.2.1.391-459
KCFNCGKEGHIAKNCRAPRKRGCWKCGREGHQMKDCNERQANFLGKIWPSHKGRPGNFLQSRPEPTAPP

SEQ ID NO: 4 - protein, 182 aa, Artificial Sequence
  Mos.Pol.2.1.94-275 peptide
LPGKWKPKMIGGIGGFIKVKQYDQILIEICGKKAIGTVLVGPTPVNIIGRNMLTQLGCTLNFPISPIDTVPVTLKPGMDGPRVKQWPLTEEKIKALTEICKEMEKEGKITKIGPENPYNTPIFAIKKKDSTKWRKLVDFRELNKKTQDFWEVQLGIPHPAGLKKKKSVTVLDVGDAYFSVPL

SEQ ID NO: 5 - protein, 37 aa, Artificial Sequence
  Mos.Pol.2.1.363-399 peptide
HLLKWGFTTPDKKHQKEPPFLWMGYELHPDRWTVQPI

SEQ ID NO: 6 - protein, 29 aa, Artificial Sequence
  Mos.Pol.2.1.482-510 peptide
AEIQKQGQDQWTYQIYQEPFKNLKTGKYA

SEQ ID NO: 7 - protein, 58 aa, Artificial Sequence
  Mos.Pol.2.1.741-798 peptide
FNLPPIVAKEIVANCDKCQLKGEAMHGQVDCSPGIWQLDCTHLEGKVILVAVHVASGY

SEQ ID NO: 8 - protein, 152 aa, Artificial Sequence
  Mos.Pol.2.1.852-1003 peptide
QEFGIPYNPQSQGVVESMNKELKKIIGQVREQAEHLKTAVQMAVFIHNFKRKGGIGGYSAGERIIDIIATDIQTKELQKQITKIQNFRVYYRDSRDPIWKGPAKLLWKGEGAVVIQDNSDIKVVPRRKVKIIKDYGKQMAGADCVAGRQDED

SEQ ID NO: 9 - protein, 86 aa, Artificial Sequence
  Mos.Env.2.2.516-601 peptide
GFLGAAGSTMGAASLTLTVQARQLLSGIVQQQSNLLRAIEAQQHMLQLTVWGIKQLQTRVLAIERYLKDQQLLGLWGCSGKLICTT

SEQ ID NO: 10 - protein, 231 aa, Artificial Sequence
  Mos.Gag.2.2.133-363 peptide
PIVQNAQGQMVHQALSPRTLNAWVKVVEEKAFSPEVIPMFSALSEGATPQDLNMMLNIVGGHQAAMQMLKETINEEAAEWDRLHPVHAGPIPPGQMREPRGSDIAGTTSTLQEQIGWMTNNPPIPVGEIYKRWIIMGLNKIVRMYSPTSILDIKQGPKEPFRDYVDRFYKTLRAEQASQEVKNWMTETLLVQNANPDCKTILKALGPAATLEEMMTACQGVGGPSHKARVL

SEQ ID NO: 11 - protein, 69 aa, Artificial Sequence
  Mos.Gag.2.2.391-459 peptide
KCFNCGKEGHLARNCRAPRKKGCWKCGKEGHQMKDCTERQANFLGKIWPSNKGRPGNFPQSRPEPSAPP

SEQ ID NO: 12 - protein, 182 aa, Artificial Sequence
  Mos.Pol.2.2.94-275 peptide
LPGRWKPKMIGGIGGFIKVRQYDQIPIEICGHKAIGTVLIGPTPVNIIGRNLLTQIGCTLNFPISPIETVPVKLKPGMDGPKVKQWPLTEEKIKALVEICTEMEKEGKISKIGPENPYNTPVFAIKKKDSTRWRKLVDFRELNKRTQDFWEVQLGIPHPSGLKKKRSVTVLDVGDAYFSVPL

SEQ ID NO: 13 - protein, 37 aa, Artificial Sequence
  Mos.Pol.2.2.363-399 peptide
HLLRWGFTTPDKKHQKEPPFHWMGYELHPDKWTVQPI

SEQ ID NO: 14 - protein, 29 aa, Artificial Sequence
  Mos.Pol.2.2.482-510 peptide
AEIQKQGQGQWTYQIYQEPYKNLKTGKYA

SEQ ID NO: 15 - protein, 58 aa, Artificial Sequence
  Mos.Pol.2.2.741-798 peptide
FNLPPVVAKEIVASCDKCQLKGEAIHGQVDCSPGMWQLDCTHLEGKIILVAVHVASGY

SEQ ID NO: 16 - protein, 152 aa, Artificial Sequence
  Mos.Pol.2.2.852-1003 peptide
QEFGIPYNPQSQGVVESMNNELKKIIGQVRDQAEHLKTAVQMAVLIHNFKRRGGIGGYSAGERIVDIIATDIQTRELQKQIIKIQNFRVYYRDSRDPLWKGPAKLLWRGEGAVVIQDNSEIKVVPRRKAKIIRDYGKQMAGDDCVASRQDED

SEQ ID NO: 17 - protein, 333 aa, Artificial Sequence
  Mos.Pol.2.1.94-426 peptide
LPGKWKPKMIGGIGGFIKVKQYDQILIEICGKKAIGTVLVGPTPVNIIGRNMLTQLGCTLNFPISPIDTVPVTLKPGMDGPRVKQWPLTEEKIKALTEICKEMEKEGKITKIGPENPYNTPIFAIKKKDSTKWRKLVDFRELNKKTQDFWEVQLGIPHPAGLKKKKSVTVLDVGDAYFSVPLDESFRKYTAFTIPSINNETPGIRYQYNVLPQGWKGSPAIFQSSMTKILEPFRAKNPEIVIYQYMDDLYVGSDLEIGQHRAKIEELREHLLKWGFTTPDKKHQKEPPFLWMGYELHPDRWTVQPIQLPEKESWTVNDIQKLIGKLNWASQIY

SEQ ID NO: 18 - protein, 333 aa, Artificial Sequence
  Mos.Pol.2.2.94-426 peptide
LPGRWKPKMIGGIGGFIKVRQYDQIPIEICGHKAIGTVLIGPTPVNIIGRNLLTQIGCTLNFPISPIETVPVKLKPGMDGPKVKQWPLTEEKIKALVEICTEMEKEGKISKIGPENPYNTPVFAIKKKDSTRWRKLVDFRELNKRTQDFWEVQLGIPHPSGLKKKRSVTVLDVGDAYFSVPLDKDFRKYTAFTIPSTNNETPGVRYQYNVLPMGWKGSPAIFQCSMTKILEPFRKQNPDIVIYQYMDDLYIGSDLEIGQHRTKIEELRQHLLRWGFTTPDKKHQKEPPFHWMGYELHPDKWTVQPIVLPEKDSWTVNDIQKLVGKLNWASQIY

SEQ ID NO: 19 - protein, 16 aa, Artificial Sequence
  Pol peptide
KNPEIVIYQYMDDLYV

SEQ ID NO: 20 - protein, 15 aa, Artificial Sequence
  Pol peptide
VIYQYMDDLYVGSDL

SEQ ID NO: 21 - protein, 23 aa, Artificial Sequence
  tPA leader peptide
MDAMKRGLCCVLLLCGAVFVSAR

SEQ ID NO: 22 - protein, 86 aa, Artificial Sequence
  HXB2.516-601 peptide
GFLGAAGSTMGAASMTLTVQARQLLSGIVQQQNNLLRAIEAQQHLLQLTVWGIKQLQARILAVERYLKDQQLLGIWGCSGKLICTT

SEQ ID NO: 23 - protein, 231 aa, Artificial Sequence
  HXB2.133-363 peptide
PIVQNIQGQMVHQAISPRTLNAWVKVVEEKAFSPEVIPMFSALSEGATPQDLNTMLNTVGGHQAAMQMLKETINEEAAEWDRVHPVHAGPIAPGQMREPRGSDIAGTTSTLQEQIGWMTNNPPIPVGEIYKRWIILGLNKIVRMYSPTSILDIRQGPKEPFRDYVDRFYKTLRAEQASQEVKNWMTETLLVQNANPDCKTILKALGPAATLEEMMTACQGVGGPGHKARVL

SEQ ID NO: 24 - protein, 69 aa, Artificial Sequence
  HXB2.Gag.391-459 peptide
KCFNCGKEGHTARNCRAPRKKGCWKCGKEGHQMKDCTERQANFLGKIWPSYKGRPGNFLQSRPEPTAPP

SEQ ID NO: 25 - protein, 182 aa, Artificial Sequence
  HXB2.Pol.94-275 peptide
LPGRWKPKMIGGIGGFIKVRQYDQILIEICGHKAIGTVLVGPTPVNIIGRNLLTQIGCTLNFPISPIETVPVKLKPGMDGPKVKQWPLTEEKIKALVEICTEMEKEGKISKIGPENPYNTPVFAIKKKDSTKWRKLVDFRELNKRTQDFWEVQLGIPHPAGLKKKKSVTVLDVGDAYFSVPL

SEQ ID NO: 26 - protein, 37 aa, Artificial Sequence
  HXB2.Pol.363-399 peptide
HLLRWGLTTPDKKHQKEPPFLWMGYELHPDKWTVQPI

SEQ ID NO: 27 - protein, 29 aa, Artificial Sequence
  HXB2.Pol.482-510 peptide
AEIQKQGQGQWTYQIYQEPFKNLKTGKYA

SEQ ID NO: 28 - protein, 58 aa, Artificial Sequence
  HXB2.Pol.741-798 peptide
FNLPPVVAKEIVASCDKCQLKGEAMHGQVDCSPGIWQLDCTHLEGKVILVAVHVASGY

SEQ ID NO: 29 - protein, 152 aa, Artificial Sequence
  HXB2.Pol.852-1003 peptide
QEFGIPYNPQSQGVVESMNKELKKIIGQVRDQAEHLKTAVQMAVFIHNFKRKGGIGGYSAGERIVDIIATDIQTKELQKQITKIQNFRVYYRDSRNPLWKGPAKLLWKGEGAVVIQDNSDIKVVPRRKAKIIRDYGKQMAGDDCVASRQDED

SEQ ID NO: 30 - protein, 332 aa, Artificial Sequence
  HXB2.Pol.94-426 peptide
LPGRWKPKMIGGIGGFIKVRQYDQILIEICGHKAIGTVLVGPTPVNIIGRNLLTQIGCTLNFPISPIETVPVKLKPGMDGPKVKQWPLTEEKIKALVEICTEMEKEGKISKIGPENPYNTPVFAIKKKDSTKWRKLVDFRELNKRTQDFWEVQLGIPHPAGLKKKKSVTVLDVGDAYFSVPLDEDFRKYTAFTIPSINNETPGIRYQYNVLPQGWKGSPAIFQSSMTKILEPFRKQNPDIVIYQYMDDLYVGSDLEIGQHRTKIEELRQHLLRWGLTTPDKKHQKEPPFLWMGYELHPDKWTVQPIVLPEKDSWTVNDIQKLVGKLNWASQI

SEQ ID NO: 31 - protein, 86 aa, Artificial Sequence
  Mcon.Env.516-601 peptide
GFLGAAGSTMGAASITLTVQARQLLSGIVQQQSNLLRAIEAQQHLLQLTVWGIKQLQARVLAVERYLKDQQLLGIWGCSGKLICTT

SEQ ID NO: 32 - protein, 231 aa, Artificial Sequence
  Mcon.Gag.133-363 peptide
PIVQNLQGQMVHQAISPRTLNAWVKVVEEKAFSPEVIPMFSALSEGATPQDLNTMLNTVGGHQAAMQMLKDTINEEAAEWDRLHPVHAGPIPPGQMREPRGSDIAGTTSTLQEQIGWMTSNPPIPVGEIYKRWIILGLNKIVRMYSPVSILDIRQGPKEPFRDYVDRFFKTLRAEQATQDVKNWMTDTLLVQNANPDCKTILKALGPGATLEEMMTACQGVGGPSHKARVL

SEQ ID NO: 33 - protein, 69 aa, Artificial Sequence
  Mcon.Gag.391-459 peptide
KCFNCGKEGHIARNCRAPRKKGCWKCGKEGHQMKDCTERQANFLGKIWPSNKGRPGNFLQSRPEPTAPP

SEQ ID NO: 34 - protein, 182 aa, Artificial Sequence
  Mcon.Pol.94-275 peptide
LPGKWKPKMIGGIGGFIKVRQYDQILIEICGKKAIGTVLVGPTPVNIIGRNMLTQIGCTLNFPISPIETVPVKLKPGMDGPKVKQWPLTEEKIKALTEICTEMEKEGKISKIGPENPYNTPIFAIKKKDSTKWRKLVDFRELNKRTQDFWEVQLGIPHPAGLKKKKSVTVLDVGDAYFSVPL

SEQ ID NO: 35 - protein, 37 aa, Artificial Sequence
  Mcon.Pol.363-399 peptide
HLLRWGFTTPDKKHQKEPPFLWMGYELHPDKWTVQPI

SEQ ID NO: 36 - protein, 29 aa, Artificial Sequence
  Mcon.Pol.482-510 peptide
AEIQKQGQDQWTYQIYQEPFKNLKTGKYA

SEQ ID NO: 37 - protein, 58 aa, Artificial Sequence
  Mcon.Pol.741-798 peptide
FNLPPIVAKEIVASCDKCQLKGEAMHGQVDCSPGIWQLDCTHLEGKIILVAVHVASGY

SEQ ID NO: 38 - protein, 152 aa, Artificial Sequence
  Mcon.Pol.852-1003 peptide
QEFGIPYNPQSQGVVESMNKELKKIIGQVRDQAEHLKTAVQMAVFIHNFKRKGGIGGYSAGERIIDIIATDIQTKELQKQITKIQNFRVYYRDSRDPIWKGPAKLLWKGEGAVVIQDNSEIKVVPRRKAKIIRDYGKQMAGDDCVAGRQDED

SEQ ID NO: 39 - protein, 333 aa, Artificial Sequence
  Mcon.Pol.94-426 peptide
LPGKWKPKMIGGIGGFIKVRQYDQILIEICGKKAIGTVLVGPTPVNIIGRNMLTQIGCTLNFPISPIETVPVKLKPGMDGPKVKQWPLTEEKIKALTEICTEMEKEGKISKIGPENPYNTPIFAIKKKDSTKWRKLVDFRELNKRTQDFWEVQLGIPHPAGLKKKKSVTVLDVGDAYFSVPLDEDFRKYTAFTIPSINNETPGIRYQYNVLPQGWKGSPAIFQSSMTKILEPFRTQNPEIVIYQYMDDLYVGSDLEIGQHRTKIEELREHLLRWGFTTPDKKHQKEPPFLWMGYELHPDKWTVQPIQLPEKDSWTVNDIQKLVGKLNWASQIY